European Patent Specification EP 3 233 917 B1, published April 17, 2024. Title: Fusion protein comprising three binding domains to 5T4 and CD3. Applicant: Biotechnol Llimited. The sequence listing filed with the application follows.

SEQUENCE LISTING (52 sequences)

SEQ ID NO: 1 - protein, 120 aa, Artificial
  Artificial sequence part of the fusion protein
EVQLQQSGPDLVKPGASVKISCKASGYSFTGYYMHWVKQSHGKSLEWIGRINPNNGVTLYNQKFKDKAILTVDKSSTTAYMELRSLTSEDSAVYYCARSTMITNYVMDYWGVTTSVTVSS

SEQ ID NO: 2 - protein, 120 aa, Artificial
  Artificial sequence part of the fusion protein
EVQLQQSGPDLVKPGASVKISCKASGYSFTGYYMHWVKQSPGKGLEWIGRINPNNGVTLYNQKFKDKATLTVDKSSTTAYMELRSLTSEDSAVYYCARSTMITNYVMDYWGQGTSVTVSS

SEQ ID NO: 3 - protein, 120 aa, Artificial
  Artificial sequence part of the fusion protein
QVQLVQSGAEVKKPGASVKVSCKASGYSFTGYYMHWVKQSPGQGLEWIGRINPNNGVTLYNQKFKDRVTMTRDTSISTAYMELSRLRSDDTAVYYCARSTMITNYVMDYWGQGTLVTVSS

SEQ ID NO: 4 - protein, 120 aa, Artificial
  Artificial sequence part of the fusion protein
QVQLVQSGAEVKKPGASVKVSCKASGYSFTGYYMHWVRQAPGQGLEWMGRINPNNGVTLYNQKFKDRVTMTRDTSISTAYMELSRLRSDDTAVYYCARSTMITNYVMDYWGQGTLVTVSS

SEQ ID NO: 5 - protein, 120 aa, Artificial
  Artificial sequence part of the fusion protein
QVQLVQSGAEVKKPGASVKVSCKASGYSFTGYYMHWVRQAPGQGLEWMGRINPNNGVTLYNQKFKDRVTITRDTSTSTAYMELSSLRSEDTAVYYCARSTMITNYVMDYWGQGTLVTVSS

SEQ ID NO: 6 - protein, 120 aa, Artificial
  Artificial sequence part of the fusion protein
QVQLVQSGAEVKKPGASVKVSCKASGYSFTSYYMHWVKQSPGQGLEWIGRINPNNGVTLYNQKFKDRVTMTRDTSISTAYMELSRLRSDDTAVYYCARSTMITNYVMDYWGQGTLVTVSS

SEQ ID NO: 7 - protein, 120 aa, Artificial
  Artificial sequence part of the fusion protein
QVQLVQSGAEVKKPGASVKVSCKASGYSFTGYYMHWVKQSPGQGLEWIGWINPNSGGTNYAQKFQGRVTMTRDTSISTAYMELSRLRSDDTAVYYCARSTMITNYVMDYWGQGTLVTVSS

SEQ ID NO: 8 - protein, 120 aa, Artificial
  Artificial sequence part of the fusion protein
QVQLVQSGSELKKPGASVKVSCKASGYSFTGYYMHWVRQAPGQGLEWMGRINPNNGVTLYNQKFKDKFVFSLDTSVSTAYLQICSLKAEDTAVYYCARSTMITNYVMDYWGQGTLVTVSS

SEQ ID NO: 9 - protein, 120 aa, Artificial
  Artificial sequence part of the fusion protein
QVQLVQSGAEVKKPGASVKVSCKVSGYSFTGYYMHWVRQAPGKGLEWMGRINPNNGVTLYNQKFKDKVTMTEDTSTDTAYMELSSLRSEDTAVYYCATSTMITNYVMDYWGQGTLVTVSS

SEQ ID NO: 10 - protein, 120 aa, Artificial
  Artificial sequence part of the fusion protein
QMQLVQSGPEVKKPGTSVKVSCKASGYSFTGYYMHWVRQARGQRLEWIGRINPNNGVTLYNQKFKDKVTITRDMSTSTAYMELSSLRSEDTAVYYCAASTMITNYVMDYWGQGTLVTVSS

SEQ ID NO: 11 - protein, 120 aa, Artificial
  Artificial sequence part of the fusion protein
QVQLVQSGAEVKKPGASVKVSCKASGYSFTGYYMHWVRQAPGQRLEWMGRINPNNGVTLYNQKFKDKVTITRDTSASTAYMELSSLRSEDTAVYYCARSTMITNYVMDYWGQGTLVTVSS

SEQ ID NO: 12 - protein, 120 aa, Artificial
  Artificial sequence part of the fusion protein
QVQLVQSGAEVKKPGSSVKVSCKASGYSFTGYYMHWVRQAPGQGLEWMGRINPNNGVTLYNQKFKDKVTITADKSTSTAYMELSSLRSEDTAVYYCARSTMITNYVMDYWGQGTLVTVSS

SEQ ID NO: 13 - protein, 120 aa, Artificial
  Artificial sequence part of the fusion protein
QVQLVQSGSELKKPGASVKVSCKASGYSFTGYYMHWVRQAPGQGLEWMGRINPNNGVTLYNQKFKDKVTITADKSTSTAYMELSSLRSEDTAVYYCARSTMITNYVMDYWGQGTLVTVSS

SEQ ID NO: 14 - protein, 120 aa, Artificial
  Artificial sequence part of the fusion protein
QVKLQQSGPGLVTPSQSLSITCTVSGYSFTGYYMHWVRQSPGQGLEWLGRINPNNGVTLYNQKFKDKKSISKDNSKSQVFLKMNSLQADDTAVYYCARSTMITNYVMDYWGQGTTVTVSS

SEQ ID NO: 15 - protein, 120 aa, Artificial
  Artificial sequence part of the fusion protein
QVQLQESGPGLVKPSQTLSLTCTVSGYSFTGYYMHWVRQPPGKGLEWIGRINPNNGVTLYNQKFKDKVTISVDTSKNQFSLKLSSVTAADTAVYYCARSTMITNYVMDYWGQGTLVTVSS

SEQ ID NO: 16 - protein, 107 aa, Artificial
  Artificial sequence part of the fusion protein
DIVMTQTPTFLLVSACDRVTITCKASQSVSNDVAWYQQKPGQSPTLLISYTSSRYAGVPDRFIGSGYGTDFTFTISTLQAEDLAVYFCQQDYNSPPTFGGGTKLEIK

SEQ ID NO: 17 - protein, 108 aa, Artificial
  Artificial sequence part of the fusion protein
ASIVMTQTPTSLLVSAGDRVTITCKASQSVSNDVAWYQQKPGQSPKLLISYTSSRYAGVPDRFSGSGYGTDFTLTISSVQAEDAAVYFCQQDYNSPPTFGGGTKLEIK

SEQ ID NO: 18 - protein, 107 aa, Artificial
  Artificial sequence part of the fusion protein
DIVMTQSPDSLAVSLGERATINCKASQSVSNDVAWYQQKPGQSPKLLISYTSSRYAGVPDRFSGSGSGTDFTLTISSLQAEDVAVYFCQQDYNSPPTFGGGTKLEIK

SEQ ID NO: 19 - protein, 107 aa, Artificial
  Artificial sequence part of the fusion protein
DIVMTQSPDSLAVSLGERATINCKASQSVSNDVAWYQQKPGQPPKLLIYYTSSRYAGVPDRFSGSGSGTDFTLTISSLQAEDVAVYYCQQDYNSPPTFGGGTKLEIK

SEQ ID NO: 20 - protein, 107 aa, Artificial
  Artificial sequence part of the fusion protein
DIVMTQSPDSLAVSLGERATINCRASQGIRNDLGWYQQKPGQPPKLLIYYTSSRYAGVPDRFSGSGSGTDFTLTISSLQAEDVAVYYCQQDYNSPPTFGGGTKLEIK

SEQ ID NO: 21 - protein, 107 aa, Artificial
  Articial sequence part of the fusion protein
DIVMTQSPDSLAVSLGERATINCKASQSVSNDVAWYQQKPGQPPKLLIYAASSLQSGVPDRFSGSGSGTDFTLTISSLQAEDVAVYYCQQDYNSPPTFGGGTKLEIK

SEQ ID NO: 22 - protein, 107 aa, Artificial
  Artificial sequence part of the fusion protein
DIQMTQSPSSLSASVGDRVTITCKASQSVSNDVAWYQQKPGKAPKRLIYYTSSRYAGVPSRFSGSGSGTEFTLTISSLQPEDFATYYCQQDYNSPPTFGGGTKLEIK

SEQ ID NO: 23 - protein, 107 aa, Artificial; identical to SEQ ID NO: 19
  Artificial sequence part of the fusion protein

SEQ ID NO: 24 - protein, 107 aa, Artificial
  Artificial sequence part of the fusion protein
EIVMTQSPSTLSASVGDRVIITCKASQSVSNDVAWYQQKPGKAPKLLIYYTSSRYAGVPSRFSGSGSGAEFTLTISSLQPDDFATYYCQQDYNSPPTFGQGTKLTVL

SEQ ID NO: 25 - protein, 105 aa, Artificial
  Artificial sequence part of the fusion protein
EIVLTQSPATLSLSPGERATLSCKASQSVSNDVAWYQQKPGQAPRLLIYDASNRATGIPARFSGSGPGTDFTLTISSLEPEDFAVYYCQQRSNWHFGQGTKVEIK

SEQ ID NO: 26 - protein, 119 aa, Artificial [sequence omitted]

SEQ ID NO: 27 - protein, 119 aa, Artificial
  Artificial sequence part of the fusion protein
QVQLVQSGGGVVQPGRSLRLSCKASGYTFTRYTMHWVRQAPGKGLEWIGYINPSRGYTNYNQKVKDRFTISRDNSKNTAFLQMDSLRPEDTGVYFCARYYDDHYSLDYWGQGTPVTVSS

SEQ ID NO: 28 - protein, 119 aa, Artificial
  Artificial sequence part of the fusion protein
DVQLVQSGAEVKKPGASVKVSCKASGYTFTRYTMHWVRQAPGQGLEWIGYINPSRGYTNYADSVKGRFTITTDKSTSTAYMELSSLRSEDTATYYCARYYDDHYCLDYWGQGTTVTVSS

SEQ ID NO: 29 - protein, 119 aa, Artificial
  Artificial sequence part of the fusion protein
QVQLVQSGAELKKPGASVKVSCKASGYTFTRYTMHWVRQAPGQCLEWMGYINPSRGYTNYNQKFKDKATLTADKSTSTAYMELRSLRSDDTAVYYCARYYDDHYSLDYWGQGTLVTVSS

SEQ ID NO: 30 - protein, 118 aa, Artificial [sequence omitted]

SEQ ID NO: 31 - protein, 114 aa, Artificial
  Artificial sequence part of the fusion protein
QVQLQQSGAELARPGASVKMSCKASGYTFTSYTMHWVKQRPGQGLEWIGYINPSSGYTKYNQKFKDKATLTADKSSSTAYHQLSSLTSEDSAVYYCARWQDYDVYFDYWGQGTT

SEQ ID NO: 32 - protein, 122 aa, Artificial
  Artificial sequence part of the fusion protein
EVQLVESGGGLVQPGGSLRLSCAASGYSFTGYTMNWVRQAPGKGLEWVALINPYKGVTTYADSVKGRFTISVDKSKNTAYLQMNSLRAEDTAVYYCARSGYYGDSDWYFDVWGQGTLVTVSS

SEQ ID NO: 33 - protein, 120 aa, Artificial
  Artificial sequence part of the fusion protein
QVQLQQSGAELARPGASVKMSCKASGYTFISYTMHWVKQRPGQGLEWIGYINPRSGYTHYNQKLKDKATLTADKSSSSAYMQLSSLTSEDSAVYYCARSAYYDYDGFAYWGQGTLVTVSA

SEQ ID NO: 34 - protein, 106 aa, Artificial [sequence omitted]

SEQ ID NO: 35 - protein, 106 aa, Artificial [sequence omitted]

SEQ ID NO: 36 - protein, 106 aa, Artificial
  Artificial sequence parr of the fusion protein
DIQMTQSPSSLSASVGDRVTITCRASQSVSYMNWYQQKPGKAPKRWIYDTSKVASGVPARFSGSGSGTDYSLTINSLEAEDAATYYCQQWSSNPLTFGGGTKVEIK

SEQ ID NO: 37 - protein, 108 aa, Artificial
  Artificial sequence part of the fusion protein
DIQLTQSPSILSASVGDRVTITCRASSSVSYMNWYQQKPGKAPKRWIYDTSKVASGVPYRFSGSGSGTEYTLTISSMQPEDFATYYCQQWSSNPLTFGCGTKVEIKRT

SEQ ID NO: 38 - protein, 108 aa, Artificial [sequence omitted]

SEQ ID NO: 39 - protein, 104 aa, Artificial
  Artificial sequence part of the fusion protein
QIVLSQSPALLSASPGEKVTMTCRASSSYMHWYQQKPGSSPKPWIYATSNLASGVPARFSGSGSGTSYSLTISRVEAEDAATYYCQQWSSNPPTFGGGTKLETK

SEQ ID NO: 40 - protein, 107 aa, Artificial [sequence omitted]

SEQ ID NO: 41 - protein, 106 aa, Artificial
  Artificial sequence part of the fusion protein
QIVLTQSPAIMSASPGEKVTMTCSASSSVSYMNWYKQKSGTSPKRWTYDTSKLASGVPARFSGSGSGTSYSLTISSMEAEDAATYYCQQWSSNPPTFGSGTKLEIK

SEQ ID NO: 42 - protein, 247 aa, Artificial
  Combined VH/VL
EVQLQQSGPDLVKPGASVKISCKASGYSFTGYYMHWVKQSPGKGLEWIGRINPNNGVTLYNQKFKDKATLTVDKSSTTAYMELRSLTSEDSAVYYCARSTMITNYVMDYWGQGTSVTVSSASGGGGSGGGGSGGGGSAGASIVMTQTPTSLLVSAGDRVTITCKASQSVSNDVAWYQQKPGQSPKLLISYTSSRYAGVPDRFSGSGYGTDFTLTISSVQAEDAAVYFCQQDYNSPPTFGGGTKLEIK

SEQ ID NO: 43 - protein, 246 aa, Artificial
  Combined VH/VL
QVQLVQSGAEVKKPGASVKVSCKASGYSFTGYYMHWVKQSPGQGLEWIGRINPNNGVTLYNQKFKDRVTMTRDTSISTAYMELSRLRSDDTAVYYCARSTMITNYVMDYWGQGTLVTVSSASGGGGSGGGGSGGGGSAGDIVMTQSPDSLAVSLGERATINCKASQSVSNDVAWYQQKPGQPPKLLIYYTSSRYAGVPDRFSGSGSGTDFTLTISSLQAEDVAVYYCQQDYNSPPTFGGGTKLEIK

SEQ ID NO: 44 - protein, 246 aa, Artificial
  Combined VH/VL
QVQLVQSGAEVKKPGASVKVSCKASGYSFTSYYMHWVKQSPGQCLEWIGRINPNNGVTLYNQKFKDRVTMTRDTSISTAYMELSRLRSDDTAVYYCARSTMITNYVMDYWGQGTLVTVSSASGGGGSGGGGSGGGGSAGDIVMTQSPDSLAVSLGERATINCKASQSVSNDVAWYQQKPGQPPKLLIYYTSSRYAGVPDRFSGSGSGTDFTLTISSLQAEDVAVYYCQQDYNSPPTFGCGTKLEIK

SEQ ID NO: 45 - protein, 244 aa, Artificial
  Combined VH/VL
QVQLQQSGAELARPGASVKMSCKASGYTFTRYTMHWVKQRPGQGLEWIGYINPSRGYTNYNQKFKDKATLTTDKSSSTAYMQLSSLTSEDSAVYYCARYYDDHYCLDYWGQGTTLTVSSASGGGGSGGGGSGGGGSAGQIVLTQSPAIMSASPGEKVTMTCSASSSVSYMNWYQQKSGTSPKRWIYDTSKLASGVPAHFRGSGSGTSYSLTISGMEAEDAATYYCQQWSSNPFTFGSGTKLEIN

SEQ ID NO: 46 - protein, 244 aa, Artificial
  Combined VH/VL
QVQLVQSGAELKKPGASVKVSCKASGYTFTRYTMHWVRQAPGQGLEWMGYINPSRGYTNYNQKFKDKATLTADKSTSTAYMELRSLRSDDTAVYYCARYYDDHYSLDYWGQGTLVTVSSASGGGGSGGGGSGGGGSAGDIQLTQSPSILSASVGDRVTITCRASSSVSYMNWYQQKPGKAPKRWIYDTSKVASGVPYRFSGSGSGTEYTLTISSMQPEDFATYYCQQWSSNPLTFGGGTKVEIK

SEQ ID NO: 47 - protein, 244 aa, Artificial
  Combined VH/VL
QVQLVQSGAELKKPGASVKVSCKASGYTFTRYTMHWVRQAPGQCLEWMGYINPSRGYTNYNQKFKDKATLTADKSTSTAYMELRSLRSDDTAVYYCARYYDDHYSLDYWGQGTLVTVSSASGGGGSGGGGSGGGGSAGDIQLTQSPSILSASVGDRVTITCRASSSVSYMNWYQQKPGKAPKRWIYDTSKVASGVPYRFSGSGSGTEYTLTISSMQPEDFATYYCQQWSSNPLTFGCGTKVEIK

SEQ ID NO: 48 - protein, 248 aa, Artificial
  Combined VH/VL
EVQLVESGGGLVQPGGSLRLSCAASGYSFTGYTMNWVRQAPGKCLEWVALINPYKGVTTYADSVKGRFTISVDKSKNTAYLQMNSLRAEDTAVYYCARSGYYGDSDWYFDVWGQGTLVTVSSASGGGGSGGGGSGGGGSAGDIQMTQSPSSLSASVGDRVTITCRASQDIRNYLNWYQQKPGKAPKLLIYYTSRLESGVPSRFSGSGSGTDYTLTISSLQPEDFATYYCQQGNTLPWTFGCGTKVEIK

SEQ ID NO: 49 - protein, 480 aa, Artificial
  CH1 containing chain of Tb535c
EVQLQQSGPDLVKPGASVKISCKASGYSFTGYYMHWVKQSPGKGLEWIGRINPNNGVTLYNQKFKDKATLTVDKSSTTAYMELRSLTSEDSAVYYCARSTMITNYVMDYWGQGTSVTVSSASTKGPSVFPLAPSSKSTSGGTAALGCLVKDYFPEPVTVSWNSGALTSGVHTFPAVLQSSGLYSLSSVVTVPSSSLGTQTYICNVNHKPSNTKVDKKVEPKSCDKTHTGPGGGSPGQVQLVQSGAELKKPGASVKVSCKASGYTFTRYTMHWVRQAPGQCLEWMGYINPSRGYTNYNQKFKDKATLTADKSTSTAYMELRSLRSDDTAVYYCARYYDDHYSLDYWGQGTLVTVSSASGGGGSGGGGSGGGGSAGDIQLTQSPSILSASVGDRVTITCRASSSVSYMNWYQQKPGKAPKRWIYDTSKVASGVPYRFSGSGSGTEYTLTISSMQPEDFATYYCQQWSSNPLTFGCGTKVEIK

SEQ ID NO: 50 - protein, 470 aa, Artificial
  CL containing chain of Tb535c
SIVMTQTPTSLLVSAGDRVTITCKASQSVSNDVAWYQQKPGQSPKLLISYTSSRYAGVPDRFSGSGYGTDFTLTISSVQAEDAAVYFCQQDYNSPPTFGGGTKLEIKRTVAAPSVFIFPPSDEQLKSGTASVVCLLNNFYPREAKVQWKVDNALQSGNSQESVTEQDSKDSTYSLSSTLTLSKADYEKHKVYACEVTHQGLSSPVTKSFNRGECGPGGGSPGEVQLVQSGPDDVKPGGSVKISCKASGYSFTGYYMHWVKQSPGKCLEWIGRINPNNGVTLYNQKFKDKATLTVDKSSTTAYMELRSLTSEDSAVYYCARSTMITNYVMDYWGQGTLVTVSSASGGGGSGGGGSGGGGSAGDIVMTQTPTSLLVSAGDRVTITCKASQSVSNDVAWYQQKPGQSPKLLISYTSSRYAGVPDRFSGSGYGTDFTLTISSVQAEDAAVYFCQQDYNSPPTFGCGTKLEIKSG

SEQ ID NO: 51 - protein, 482 aa, Artificial
  CH1 containing chain of Tb535h
QVQLVQSGAEVKKPGASVKVSCKASGYSFTSYYMHWVKQSPGQGLEWIGRINPNNGVTLYNQKFKDRVTMTRDTSISTAYMELSRLRSDDTAVYYCARSTMITNYVMDYWGQGTLVTVSSASTKGPSVFPLAPSSKSTSGGTAALGCLVKDYFPEPVTVSWNSGALTSGVHTFPAVLQSSGLYSLSSVVTVPSSSLGTQTYICNVNHKPSNTKVDKKVEPKSCDKTHTGPGGGSPGQVQLVQSGAELKKPGASVKVSCKASGYTFTRYTMHWVRQAPGQCLEWMGYINPSRGYTNYNQKFKDKATLTADKSTSTAYMELRSLRSDDTAVYYCARYYDDHYSLDYWGQGTLVTVSSASGGGGSGGGGSGGGGSAGDIQLTQSPSILSASVGDRVTITCRASSSVSYMNWYQQKPGKAPKRWIYDTSKVASGVPYRFSGSGSGTEYTLTISSMQPEDFATYYCQQWSSNPLTFGCGTKVEIKSG

SEQ ID NO: 52 - protein, 470 aa, Artificial
  CL containing chain of Tb535h
DIVMTQSPDSLAVSLGERATINCKASQSVSNDVAWYQQKPGQPPKLLIYYTSSRYAGVPDRFSGSGSGTDFTLTISSLQAEDVAVYYCQQDYNSPPTFGGGTKLEIKRTVAAPSVFIFPPSDEQLKSGTASVVCLLNNFYPREAKVQWKVDNALQSGNSQESVTEQDSKDSTYSLSSTLTLSKADYEKHKVYACEVTHQGLSSPVTKSFNRGECGPGGGSPGQVQLVQSGAEVKKPGASVKVSCKASGYSFTSYYMHWVKQSPGQCLEWIGRINPNNGVTLYNQKFKDRVTMTRDTSISTAYMELSRLRSDDTAVYYCARSTMITNYVMDYWGQGTLVTVSSASGGGGSGGGGSGGGGSAGDIVMTQSPDSLAVSLGERATINCKASQSVSNDVAWYQQKPGQPPKLLIYYTSSRYAGVPDRFSGSGSGTDFTLTISSLQAEDVAVYYCQQDYNSPPTFGCGTKLEIKSG